European Patent Specification EP 4 149 957 B1, published July 3, 2024. Title: PROCEDE DE PRODUCTION D'OLIGOSACCHARIDES. Applicant: Institut National des Sciences Appliquées de Toulouse Centre national de la recherche scientifique Université Toulouse III - Paul Sabatier Institut national de la recherche pour l'agriculture, l'alimentation et l'environnement. The sequence listing filed with the application follows.

SEQUENCE LISTING (66 sequences)

SEQ ID NO: 1 - DNA, 29 bp, Artificial Sequence
  amorce PL1
ctcgagaggcgatatttttccctgtatcc

SEQ ID NO: 2 - DNA, 32 bp, Artificial Sequence
  amorce PL2
ggtttgcgtattattcagtttcaacgcgttcg

SEQ ID NO: 3 - DNA, 35 bp, Artificial Sequence
  amorce PL5
ctggagctcagaggaataatacatgtcaaaagtcg

SEQ ID NO: 4 - DNA, 29 bp, Artificial Sequence
  amorce PL6
ctcgagacaacagcgataatcacatcacc

SEQ ID NO: 5 - DNA, 32 bp, Artificial Sequence
  amorce PL3
gttgaaactgaataatacgcaaaccgcctctc

SEQ ID NO: 6 - DNA, 34 bp, Artificial Sequence
  amorce PL4
atgtattattcctctgagctccagcttttgttcc

SEQ ID NO: 7 - DNA, 19 bp, Artificial Sequence
  amorce PL7
tcgaggtcattagccacca

SEQ ID NO: 8 - DNA, 33 bp, Artificial Sequence
  amorce
ctaggatccgccgaaaattgggcggtgaataac

SEQ ID NO: 9 - DNA, 30 bp, Artificial Sequence
  amorce
gtaaagcttctggtaagcagcccagagaag

SEQ ID NO: 10 - DNA, 31 bp, Artificial Sequence
  amorce
ctcaagcttgcgccgatcctgtacatcatcc

SEQ ID NO: 11 - DNA, 34 bp, Artificial Sequence
  amorce
cgtgtcgaccgttaatcctaatctgccacgcacc

SEQ ID NO: 12 - DNA, 24 bp, Artificial Sequence
  amorce
actcgagaatggcgatgaagagag

SEQ ID NO: 13 - DNA, 19 bp, Artificial Sequence
  amorce
ccagtgccaccagttcatc

SEQ ID NO: 14 - DNA, 26 bp, Artificial Sequence
  amorce
caagcttcgattccggaagtggtgac

SEQ ID NO: 15 - DNA, 26 bp, Artificial Sequence
  amorce
aggatccatgcccccatgacaaacag

SEQ ID NO: 16 - DNA, 25 bp, Artificial Sequence
  amorce
ggatccaggcgtcggggatatcgtg

SEQ ID NO: 17 - DNA, 31 bp, Artificial Sequence
  amorce
aagcttcggtcttcatacagacccagatagc

SEQ ID NO: 18 - DNA, 26 bp, Artificial Sequence
  amorce
aagcttggccattgccgggggctgtg

SEQ ID NO: 19 - DNA, 27 bp, Artificial Sequence
  amorce
ctcgagccaccgtgtgactgacgaatc

SEQ ID NO: 20 - DNA, 31 bp, Artificial Sequence
  amorce
ttgtcgacttaaggagggcatcatgcctgac

SEQ ID NO: 21 - DNA, 29 bp, Artificial Sequence
  amorce
gttctagatgactgcaagaggtggcttcc

SEQ ID NO: 22 - DNA, 8217 bp, Artificial Sequence
  séquence plasmidique pWKS-GalP
agatctcacatgttctttcctgcgttatcccctgattctgtggataaccgtattaccgcctttgagtgagctgataccgctcgccgcagccgaacgaccgagcgcagcgagtcagtgagcgaggaagcggaagagcgcccaatacgcaaaccgcctctccccgcgcgttggccgattcattaatgcagctggcacgacaggtttcccgactggaaagcgggcagtgagcgcaacgcaattaatgtgagttagctcactcattaggcaccccaggctttacactttatgctcccggctcgtatgttgtgtggaattgtgagcggataacaatttcacacaggaaacagctatgaccatgattacgccaagcgcgcaattaaccctcactaaagggaacaaaagctgggtaccgggccccccctcgaggtcgacttaaggagggcatcatgcctgacgctaaaaaacaggggcggtcaaacaaggcaatgacgtttttcgtctgcttccttgccgctctggcgggattactctttggcctggatatcggtgtaattgctggcgcactgccgtttattgcagatgaattccagattacttcgcacacgcaagaatgggtcgtaagctccatgatgttcggtgcggcagtcggtgcggtgggcagcggctggctctcctttaaactcgggcgcaaaaagagcctgatgatcggcgcaattttgtttgttgccggttcgctgttctctgcggctgcgccaaacgttgaagtactgattctttcccgcgttctactggggctggcggtgggtgtggcctcttataccgcaccgctgtacctctctgaaattgcgccggaaaaaattcgtggcagtatgatctcgatgtatcagttgatgatcactatcgggatcctcggtgcttatctttctgataccgccttcagctacaccggtgcatggcgctggatgctgggtgtgattatcatcccggcaattttgctgctgattggtgtcttcttcctgccagacagcccacgttggtttgccgccaaacgccgttttgttgatgccgaacgcgtgctgctacgcctgcgtgacaccagcgcggaagcgaaacgcgaactggatgaaatccgtgaaagtttgcaggttaaacagagtggctgggcgctgtttaaagagaacagcaacttccgccgcgcggtgttccttggcgtactgttgcaggtaatgcagcaattcaccgggatgaacgtcatcatgtattacgcgccgaaaatcttcgaactggcgggttataccaacactaccgagcaaatgtgggggaccgtgattgtcggcctgaccaacgtacttgccacctttatcgcaatcggccttgttgaccgctggggacgtaaaccaacgctaacgctgggcttcctggtgatggctgctggcatgggcgtactcggtacaatgatgcatatcggtattcactctccgtcggcgcagtatttcgccatcgccatgctgctgatgtttattgtcggttttgccatgagtgccggtccgctgatttgggtactgtgctccgaaattcagccgctgaaaggccgcgattttggcatcacctgctccactgccaccaactggattgccaacatgatcgttggcgcaacgttcctgaccatgctcaacacgctgggtaacgccaacaccttctgggtgtatgcggctctgaacgtactgtttatcctgctgacattgtggctggtaccggaaaccaaacacgtttcgctggaacatattgaacgtaatctgatgaaaggtcgtaaactgcgcgaaataggcgctcacgattaatctccccaagcttcctcccatcgcggaggaagccacctcttgcagtcatctagagcggccgccaccgcggtggagctccaattcgccctatagtgagtcgtattacgcgcgctcactggccgtcgttttacaacgtcgtgactgggaaaaccctggcgttacccaacttaatcgccttgcagcacatccccctttcgccagctggcgtaatagcgaagaggcccgcaccgatcgcccttcccaacagttgcgcagcctgaatggcgaatgggacgcgccctgtagcggcgcattaagcgcggcgggtgtggtggttacgcgcagcgtgaccgctacacttgccagcgccctagcgcccgctcctttcgctttcttcccttcctttctcgccacgttcgccggctttccccgtcaagctctaaatcgggggctccctttagggttccgatttagtgctttacggcacctcgaccccaaaaaacttgattagggtgatggttcacgtagtgggccatcgccctgatagacggtttttcgccctttgacgttggagtccacgttctttaatagtggactcttgttccaaactggaacaacactcaaccctatctcggtctattcttttgatttataagggattttgccgatttcggcctattggttaaaaaatgagctgatttaacaaaaatttaacgcgaattttaacaaaaaattccgtatggcaatgaaagacggtgagctggtgatatgggatagtgttcacccttgttacaccgttttccatgagcaaactgaaacgttttcatcgctctggagtgaataccacgacgatttccggcagtttctacacatatattcgcaagatgtggcgtgttacggtgaaaacctggcctatttccctaaagggtttattgagaatatgtttttcgtctcagccaatccctgggtgagtttcaccagttttgatttaaacgtggccaatatggacaacttcttcgcccccgttttcaccatgggcaaatattatacgcaaggcgacaaggtgctgatgccgctggcgattcaggttcatcatgccgtttgtgatggcttccatgtcggcagaatgcttaatgaattacaacagtactgcgatgagtggcagggcggggcgtaatttttttaaggcagttattggtgcccttaaacgcctggttgctacgcctgaataagtgataataagcggatgaatggcagaaattcgaaagcaaattcgacccggtcgtcggttcagggcagggtcgttaaatagccgcttatgtctattgctggtttaccggtttattgactaccggaagcagtgtgaccgtgtgcttctcaaatgcctgaggccagtttgctcaggctctccccgtggaggtaataattgacgatatgatcatttattctgcctcccagagcctgataaaaacggttagcgccggggttggatttttcagcgttccagctaaggctaaggcattcctgttcaagcgcaagccgggctataaagcgcattatcgctttacccgtgcccttatttcgatcgcactgagaaacatacagctctttaatatgcaggtaatccgggcagcgcaacggaacattcatcagtgtaaaaatggaatcaataaagccctgcgcagcgcgcagggtcagcctgaatacgcgtttaatgaccagcacagtcgtgatggcaaggtcagaatagcgctgaggtctgcctcgtgaagaaggtgttgctgactcataccaggcctgaatcgccccatcatccagccagaaagtgagggagccacggttgatgagagctttgttgtaggtggaccagttggtgattttgaacttttgctttgccacggaacggtctgcgttgtcgggaagatgcgtgatctgatccttcaactcagcaaaagttcgatttattcaacaaagccgccgtcccgtcaagtcagcgtaatgctctgccagtgttacaaccaattaaccaattctgattagaaaaactcatcgagcatcaaatgaaactgcaatttattcatatcaggattatcaataccatatttttgaaaaagccgtttctgtaatgaaggagaaaactcaccgaggcagttccataggatggcaagatcctggtatcggtctgcgattccgactcgtccaacatcaatacaacctattaatttcccctcgtcaaaaataaggttatcaagtgagaaatcaccatgagtgacgactgaatccggtgagaatggcaaaagcttatgcatttctttccagacttgttcaacaggccagccattacgctcgtcatcaaaatcactcgcatcaaccaaaccgttattcattcgtgattgcgcctgagcgagacgaaatacgcgatcgctgttaaaaggacaattacaaacaggaatcgaatgcaaccggcgcaggaacactgccagcgcatcaacaatattttcacctgaatcaggatattcttctaatacctggaatgctgttttcccggggatcgcagtggtgagtaaccatgcatcatcaggagtacggataaaatgcttgatggtcggaagaggcataaattccgtcagccagtttagtctgaccatctcatctgtaacatcattggcaacgctacctttgccatgtttcagaaacaactctggcgcatcgggcttcccatacaatcgatagattgtcgcacctgattgcccgacattatcgcgagcccatttatacccatataaatcagcatccatgttggaatttaatcgcggcctcgagcaagacgtttcccgttgaatatggctcataacaccccttgtattactgtttatgtaagcagacagttttattgttcatgatgatatatttttatcttgtgcaatgtaacatcagagattttgagacacaacgtggctttgttgaataaatcgaacttttgctgagttgaaggatcagatcacgcatcttcccgacaacgcagaccgttccgtggcaaagcaaaagttcaaaatcaccaactggtccacctacaacaaagctctcatcaaccgtggctccctcactttctggctggatgatggggcgattcaggcctggtatgagtcagcaacaccttcttcacgaggcagacctcagcgctattctgaccttgccatcacgactgtgctggtcattaaacgcgtattcaggctgaccctgcgcgctgcgcagggctttattgattccatttttacactgatgaatgttccgttgcgctgcccggattacagctgttcgggggttcactgacgctgcgtgactacgatggtcaggttgcggaggctatggccctggtacgagcgctgaacaaaatgacgaaagcaggtatgcctgaaagcgtgcgtattgcctgaaaacacaacccgctacgggggagacttacccgaaatctgatttattcaacaaagccactttcagtatggatttgggtgttacgggggggggttggtgcttaaaatcgcgctgaggatttctgatggtgttaagcgggcggttttgagatgtaaactcgcccgtttaacataatggatcttgcgcgcaccgcccgaacaccactcgccacaaaaaaccgccggaacgtccaaaagtacgggttttgctgcccgcaaacgggctgttctggtgttgctagtttgttatcagaatcgcagatccggcttcagccggtttgccggctgaaagcgctatttcttccagaattgccatgattttttccccacgggaggcgtcactggctcccgtgttgtcggcagctttgattcgataagcagcatcgcctgtttcaggctgtctatgtgtgactgttgagctgtaacaagttgtctcaggtgttcaatttcatgttctagttgctttgttttactggtttcacctgttctattaggtgttacatgctgttcatctgttacattgtcgatctgttcatggtgaacagctttgaatgcaccaaaaactcgtaaaagctctgatgtatctatcttttttacaccgttttcatctgtgcatatggacagttttccctttgatatgtaacggtgaacagttgttctacttttgtttgttagtcttgatgcttcactgatagatacaagagccataagaacctcagatccttccgtatttagccagtatgttctctagtgtggttcgttgtttttgcgtgagccatgagaacgaaccattgagatcatacttactttgcatgtcactcaaaaattttgcctcaaaactggtgagctgaatttttgcagttaaagcatcgtgtagtgtttttcttagtccgttatgtaggtaggaatctgatgtaatggttgttggtattttgtcaccattcatttttatctggttgttctcaagttcggttacgagatccatttgtctatctagttcaacttggaaaatcaacgtatcagtcgggcggcctcgcttatcaaccaccaatttcatattgctgtaagtgtttaaatctttacttattggtttcaaaacccattggttaagccttttaaactcatggtagttattttcaagcattaacatgaacttaaattcatcaaggctaatctctatatttgccttgtgagttttcttttgtgttagttcttttaataaccactcataaatcctcatagagtatttgttttcaaaagacttaacatgttccagattatattttatgaatttttttaactggaaaagataaggcaatatctcttcactaaaaactaattctaatttttcgcttgagaacttggcatagtttgtccactggaaaatctcaaagcctttaaccaaaggattcctgatttccacagttctcgtcatcagctctctggttgctttagctaatacaccataagcattttccctactgatgttcatcatctgagcgtattggttataagtgaacgataccgtccgttctttccttgtagggttttcaatcgtggggttgagtagtgccacacagcataaaattagcttggtttcatgctccgttaagtcatagcgactaatcgctagttcatttgctttgaaaacaactaattcagacatacatctcaattggtctaggtgattttaatcactataccaattgagatgggctagtcaatgataattactagtccttttcctttgagttgtgggtatctgtaaattctgctagacctttgctggaaaacttgtaaattctgctagaccctctgtaaattccgctagacctttgtgtgttttttttgtttatattcaagtggttataatttatagaataaagaaagaataaaaaaagataaaaagaatagatcccagccctgtgtataactcactactttagtcagttccgcagtattacaaaaggatgtcgcaaacgctgtttgctcctctacaaaacagaccttaaaaccctaaaggcttaagtagcaccctcgcaagctcgggcaaatcgctgaatattccttttgtctccgaccatcaggcacctgagtcgctgtctttttcgtgacattcagttcgctgcgctcacggctctggcagtgaatgggggtaaatggcactacaggcgccttttatggattcatgcaaggaaactacccataatacaagaaaagcccgtcacgggcttctcagggcgttttatggcgggtctgcggagtggtgaatccgttagcgaggtgccgccggcttccattcaggtcgaggtggcccggctccatgcaccgcgacgcaacgcggggaggcagacaaggtatagggcggcgcctacaatccatgccaacccgttccatgtgctcgccgaggcggcataaatcgccgtgacgatcagcggtccaatgatcgaagttaggctggtaagagccgcgagcgatccttgaagctgtccctgatggtcgtcatctacctgcctggacagcatggcctgcaacgcgggcatcccgatgccgccggaagcgagaagaatcataatggggaaggccatccagcctcgcgtcgcgaacgccagcaagacgtagcccagcgcgtcggccgccatgccggcgataatggcctgcttctcgccgaaacgtttggtggcgggaccagtgacgaaggcttgagcgagggcgtgcaagattccgaataccgcaagcgacaggccgatcatcgtcgcgctccagcgaaagcggtcctcgccgaaaatgacccagagcgctgccggcacctgtcctacgagttgcatgataaagaagacagtcataagtgcggcgacgatagtcatgccccgcgcccaccggaaggagctgactgggttgaaggctctcaagggcatcggtcg

SEQ ID NO: 23 - DNA, 25 bp, Artificial Sequence
  amorce ptsG FW
cttctctcagtgggctgcttaccag

SEQ ID NO: 24 - DNA, 26 bp, Artificial Sequence
  amorce ptsG RV
ccgttaatcctaatctgccacgcacc

SEQ ID NO: 25 - DNA, 24 bp, Artificial Sequence
  amorce manXYZ FW
tgttaggcgagcaggaaaacgtcg

SEQ ID NO: 26 - DNA, 24 bp, Artificial Sequence
  amorce manXYZ RV
accaatcacacccagagcaaccag

SEQ ID NO: 27 - DNA, 25 bp, Artificial Sequence
  amorce pfkA FW
cattttgcattccaaagttcagagg

SEQ ID NO: 28 - DNA, 26 bp, Artificial Sequence
  amorce pfkA RV
tcatcggtttcagggtaaaggaatct

SEQ ID NO: 29 - DNA, 4903 bp, Artificial Sequence
  séquence plasmidique pBAD HisA comprenant le gène codant pour la protéine Teth514-1788
aagaaaccaattgtccatattgcatcagacattgccgtcactgcgtcttttactggctcttctcgctaaccaaaccggtaaccccgcttattaaaagcattctgtaacaaagcgggaccaaagccatgacaaaaacgcgtaacaaaagtgtctataatcacggcagaaaagtccacattgattatttgcacggcgtcacactttgctatgccatagcatttttatccataagattagcggatcctacctgacgctttttatcgcaactctctactgtttctccatacccgttttttgggctaacaggaggaattaaccatgggcattaaactgaaacgcctgagcgataaaccggtgttaatgccgaaagcagaaaacgagtgggaacgcgcagccgtgtttaataccgccgcaatatacgataatggtctgtttcatctgatataccgtgccaccgatattggtcctcacgccaaatatggcaaatatattagtcgcttaggctatgcagtgagtaaagatggtattaattttatgcgcctggataaaccggttatgtctaacgaaaccgaacaggaactgcgcggcttagaagatccgcgcattgtgaaaattgatggcatatattatatgatgtataccggctttggcgatcgctttcaggatgattatcgcatttgtctggccacctctaaaaatctgattgattgggaacgtaaaggcgttgtgctggatgaaccgaacaaggatgcctcactgtttccggaaaaaattaatggcaaatatgtgatgttacatcgtcgctatccggatatttggattgcctttagcgatgatctgaaaaattggtatgatcataaaccgattctgaaaccgattccgaatacctgggaatcagccagagtgggcattggcggcccgccgattaaaaccaaagatggttggtttttaatataccatgcagcagatgataataacgtgtatcgcttaggtgcagtgctgctggatctggaagatccgagcaaagttattgcacgtcagaaagaaccgattctggaaccggaactgggttgggaaaaagaaggctatattccgaatgtggtgttttcttgtggcaatgccgttaaagatgataccatatatgtgtattatggcggtgcagataccgttattggcgttgccattttagagatgaaagatattaaatttcaccatcaccatcaccattaactcgagatctgcagctggtaccatatgggaattcgaagcttggctgttttggcggatgagagaagattttcagcctgatacagattaaatcagaacgcagaagcggtctgataaaacagaatttgcctggcggcagtagcgcggtggtcccacctgaccccatgccgaactcagaagtgaaacgccgtagcgccgatggtagtgtggggtctccccatgcgagagtagggaactgccaggcatcaaataaaacgaaaggctcagtcgaaagactgggcctttcgttttatctgttgtttgtcggtgaacgctctcctgagtaggacaaatccgccgggagcggatttgaacgttgcgaagcaacggcccggagggtggcgggcaggacgcccgccataaactgccaggcatcaaattaagcagaaggccatcctgacggatggcctttttgcgtttctacaaactcttttgtttatttttctaaatacattcaaatatgtatccgctcatgagacaataaccctgataaatgcttcaataatattgaaaaaggaagagtatgagtattcaacatttccgtgtcgcccttattcccttttttgcggcattttgccttcctgtttttgctcacccagaaacgctggtgaaagtaaaagatgctgaagatcagttgggtgcacgagtgggttacatcgaactggatctcaacagcggtaagatccttgagagttttcgccccgaagaacgttttccaatgatgagcacttttaaagttctgctatgtggcgcggtattatcccgtgttgacgccgggcaagagcaactcggtcgccgcatacactattctcagaatgacttggttgagtactcaccagtcacagaaaagcatcttacggatggcatgacagtaagagaattatgcagtgctgccataaccatgagtgataacactgcggccaacttacttctgacaacgatcggaggaccgaaggagctaaccgcttttttgcacaacatgggggatcatgtaactcgccttgatcgttgggaaccggagctgaatgaagccataccaaacgacgagcgtgacaccacgatgcctgtagcaatggcaacaacgttgcgcaaactattaactggcgaactacttactctagcttcccggcaacaattaatagactggatggaggcggataaagttgcaggaccacttctgcgctcggcccttccggctggctggtttattgctgataaatctggagccggtgagcgtgggtctcgcggtatcattgcagcactggggccagatggtaagccctcccgtatcgtagttatctacacgacggggagtcaggcaactatggatgaacgaaatagacagatcgctgagataggtgcctcactgattaagcattggtaactgtcagaccaagtttactcatatatactttagattgatttaaaacttcatttttaatttaaaaggatctaggtgaagatcctttttgataatctcatgaccaaaatcccttaacgtgagttttcgttccactgagcgtcagaccccgtagaaaagatcaaaggatcttcttgagatcctttttttctgcgcgtaatctgctgcttgcaaacaaaaaaaccaccgctaccagcggtggtttgtttgccggatcaagagctaccaactctttttccgaaggtaactggcttcagcagagcgcagataccaaatactgtccttctagtgtagccgtagttaggccaccacttcaagaactctgtagcaccgcctacatacctcgctctgctaatcctgttaccagtggctgctgccagtggcgataagtcgtgtcttaccgggttggactcaagacgatagttaccggataaggcgcagcggtcgggctgaacggggggttcgtgcacacagcccagcttggagcgaacgacctacaccgaactgagatacctacagcgtgagctatgagaaagcgccacgcttcccgaagggagaaaggcggacaggtatccggtaagcggcagggtcggaacaggagagcgcacgagggagcttccagggggaaacgcctggtatctttatagtcctgtcgggtttcgccacctctgacttgagcgtcgatttttgtgatgctcgtcaggggggcggagcctatggaaaaacgccagcaacgcggcctttttacggttcctggccttttgctggccttttgctcacatgttctttcctgcgttatcccctgattctgtggataaccgtattaccgcctttgagtgagctgataccgctcgccgcagccgaacgaccgagcgcagcgagtcagtgagcgaggaagcggaagagcgcctgatgcggtattttctccttacgcatctgtgcggtatttcacaccgcatatggtgcactctcagtacaatctgctctgatgccgcatagttaagccagtatacactccgctatcgctacgtgactgggtcatggctgcgccccgacacccgccaacacccgctgacgcgccctgacgggcttgtctgctcccggcatccgcttacagacaagctgtgaccgtctccgggagctgcatgtgtcagaggttttcaccgtcatcaccgaaacgcgcgaggcagcagatcaattcgcgcgcgaaggcgaagcggcatgcataatgtgcctgtcaaatggacgaagcagggattctgcaaaccctatgctactccgtcaagccgtcaattgtctgattcgttaccaattatgacaacttgacggctacatcattcactttttcttcacaaccggcacggaactcgctcgggctggccccggtgcattttttaaatacccgcgagaaatagagttgatcgtcaaaaccaacattgcgaccgacggtggcgataggcatccgggtggtgctcaaaagcagcttcgcctggctgatacgttggtcctcgcgccagcttaagacgctaatccctaactgctggcggaaaagatgtgacagacgcgacggcgacaagcaaacatgctgtgcgacgctggcgatatcaaaattgctgtctgccaggtgatcgctgatgtactgacaagcctcgcgtacccgattatccatcggtggatggagcgactcgttaatcgcttccatgcgccgcagtaacaattgctcaagcagatttatcgccagcagctccgaatagcgcccttccccttgcccggcgttaatgatttgcccaaacaggtcgctgaaatgcggctggtgcgcttcatccgggcgaaagaaccccgtattggcaaatattgacggccagttaagccattcatgccagtaggcgcgcggacgaaagtaaacccactggtgataccattcgcgagcctccggatgacgaccgtagtgatgaatctctcctggcgggaacagcaaaatatcacccggtcggcaaacaaattctcgtccctgatttttcaccaccccctgaccgcgaatggtgagattgagaatataacctttcattcccagcggtcggtcgataaaaaaatcgagataaccgttggcctcaatcggcgttaaacccgccaccagatgggcattaaacgagtatcccggcagcaggggatcattttgcgcttcagccatacttttcatactcccgccattcagag

SEQ ID NO: 30 - DNA, 5522 bp, Artificial Sequence
  plasmide pBAD-HisA-Uhgb_MP
agaagaaaccaattgtccatattgcatcagacattgccgtcactgcgtcttttactggctcttctcgctaaccaaaccggtaaccccgcttattaaaagcattctgtaacaaagcgggaccaaagccatgacaaaaacgcgtaacaaaagtgtctataatcacggcagaaaagtccacattgattatttgcacggcgtcacactttgctatgccatagcatttttatccataagattagcggatcctacctgacgctttttatcgcaactctctactgtttctccatacccgtttttttgggctagaaataattttgtttaactttaagaaggagatatacatacccatgggatctgataaaattattcatctgactgatgattcttttgatactgatgtacttaaggcagatggtgcaatcctggttgatttctgggcacactggtgcggtccgtgcaaaatgatcgctccgattctggatgaaatcgctgacgaatatcagggcaaactgaccgttgcaaaactgaacatcgatcacaacccgggcactgcgccgaaatatggcatccgtggtatcccgactctgctgctgttcaaaaacggtgaagtggcggcaaccaaagtgggtgcactgtctaaaggtcagttgaaagagttcctcgacgctaacctggccggctctggatccggtgatgacgatgacaagctgggaattatcacaagtttgtacaaaaaagcaggctccgcggccgcccccttcaccatgagtatgagtagcaaagttattattccttgggaagaacgtccggcaggatgcaaggacgtattatggcgcagtgtggcaaaccccattattccgcgtgatttgcttcccacttccaacagtattttcaacagtgcggtagtacctttcggcgacgggtttgcaggagtattccgctgcgacgatactagccgtcgcatgcggctgcacgtagggttcagtaaagatgccataaactggaacatcaaggaagaaccgttgaagttccaatgcgatgatgaggaaatcggtacatgggtgtatggctacgacccgcgcgtgtgctttatcgaagaccgctattatgttacctggtgcaacggctatcacggtcctactatcggtgtggcctatacgttcgatttcgagacgttccaccagttggaaaacgcttttattcctttcaaccgtaacggagtacttttcccacgcaagataaacggtcgttttgccatgttgagccgtccgagcgacaatgggcatactccctttggagatattttctacagtgagtcgcccgatatggagttttggggacgccaccgccacgtgatgtcacctgccgcttttgaggtaagtgcatggcaatgcaccaaaatcggtgcaggtcctattcctgtcgagactcccgaaggctggctgctgatttatcacggtgtgctgcattcctgcaacggttatgtttacagtttcggctctgctctgctcgatttggacgaaccgtggaaggtaaagttccgctcagggccttatctgcttgccccgcgcgaaccgtacgaatgtatgggcgatgttcctaatgtatgtttcccgtgcgccgctttgcacgacaatgaaacgggcaggattgccatatactatggctgtgccgataccgtaaccggactggcattcggctatattcccgaaattatagaatttaccaaacgtacaagcatcatcaagggtgggcgcgccgacccagctttcttgtacaaagtggtgatcaagcttgaaggtaagcctatccctaaccctctcctcggtctcgattctacgcgtaccggtcatcatcaccatcaccattgagtttaaacggtctccagcttggctgttttggcggatgagagaagattttcagcctgatacagattaaatcagaacgcagaagcggtctgataaaacagaatttgcctggcggcagtagcgcggtggtcccacctgaccccatgccgaactcagaagtgaaacgccgtagcgccgatggtagtgtggggtctccccatgcgagagtagggaactgccaggcatcaaataaaacgaaaggctcagtcgaaagactgggcctttcgttttatctgttgtttgtcggtgaacgctctcctgagtaggacaaatccgccgggagcggatttgaacgttgcgaagcaacggcccggagggtggcgggcaggacgcccgccataaactgccaggcatcaaattaagcagaaggccatcctgacggatggcctttttgcgtttctacaaactctttttgtttatttttctaaatacattcaaatatgtatccgctcatgagacaataaccctgataaatgcttcaataatattgaaaaaggaagagtatgagtattcaacatttccgtgtcgcccttattcccttttttgcggcattttgccttcctgtttttgctcacccagaaacgctggtgaaagtaaaagatgctgaagatcagttgggtgcacgagtgggttacatcgaactggatctcaacagcggtaagatccttgagagttttcgccccgaagaacgttttccaatgatgagcacttttaaagttctgctatgtggcgcggtattatcccgtgttgacgccgggcaagagcaactcggtcgccgcatacactattctcagaatgacttggttgagtactcaccagtcacagaaaagcatcttacggatggcatgacagtaagagaattatgcagtgctgccataaccatgagtgataacactgcggccaacttacttctgacaacgatcggaggaccgaaggagctaaccgcttttttgcacaacatgggggatcatgtaactcgccttgatcgttgggaaccggagctgaatgaagccataccaaacgacgagcgtgacaccacgatgcctgtagcaatggcaacaacgttgcgcaaactattaactggcgaactacttactctagcttcccggcaacaattaatagactggatggaggcggataaagttgcaggaccacttctgcgctcggcccttccggctggctggtttattgctgataaatctggagccggtgagcgtgggtctcgcggtatcattgcagcactggggccagatggtaagccctcccgtatcgtagttatctacacgacggggagtcaggcaactatggatgaacgaaatagacagatcgctgagataggtgcctcactgattaagcattggtaactgtcagaccaagtttactcatatatactttagattgatttaaaacttcatttttaatttaaaaggatctaggtgaagatcctttttgataatctcatgaccaaaatcccttaacgtgagttttcgttccactgagcgtcagaccccgtagaaaagatcaaaggatcttcttgagatcctttttttctgcgcgtaatctgctgcttgcaaacaaaaaaaccaccgctaccagcggtggtttgtttgccggatcaagagctaccaactctttttccgaaggtaactggcttcagcagagcgcagataccaaatactgtccttctagtgtagccgtagttaggccaccacttcaagaactctgtagcaccgcctacatacctcgctctgctaatcctgttaccagtggctgctgccagtggcgataagtcgtgtcttaccgggttggactcaagacgatagttaccggataaggcgcagcggtcgggctgaacggggggttcgtgcacacagcccagcttggagcgaacgacctacaccgaactgagatacctacagcgtgagctatgagaaagcgccacgcttcccgaagggagaaaggcggacaggtatccggtaagcggcagggtcggaacaggagagcgcacgagggagcttccagggggaaacgcctggtatctttatagtcctgtcgggtttcgccacctctgacttgagcgtcgatttttgtgatgctcgtcaggggggcggagcctatggaaaaacgccagcaacgcggcctttttacggttcctggccttttgctggccttttgctcacatgttctttcctgcgttatcccctgattctgtggataaccgtattaccgcctttgagtgagctgataccgctcgccgcagccgaacgaccgagcgcagcgagtcagtgagcgaggaagcggaagagcgcctgatgcggtattttctccttacgcatctgtgcggtatttcacaccgcatatggtgcactctcagtacaatctgctctgatgccgcatagttaagccagtatacactccgctatcgctacgtgactgggtcatggctgcgccccgacacccgccaacacccgctgacgcgccctgacgggcttgtctgctcccggcatccgcttacagacaagctgtgaccgtctccgggagctgcatgtgtcagaggttttcaccgtcatcaccgaaacgcgcgaggcagcagatcaattcgcgcgcgaaggcgaagcggcatgcataatgtgcctgtcaaatggacgaagcagggattctgcaaaccctatgctactccgtcaagccgtcaattgtctgattcgttaccaattatgacaacttgacggctacatcattcactttttcttcacaaccggcacggaactcgctcgggctggccccggtgcattttttaaatacccgcgagaaatagagttgatcgtcaaaaccaacattgcgaccgacggtggcgataggcatccgggtggtgctcaaaagcagcttcgcctggctgatacgttggtcctcgcgccagcttaagacgctaatccctaactgctggcggaaaagatgtgacagacgcgacggcgacaagcaaacatgctgtgcgacgctggcgatatcaaaattgctgtctgccaggtgatcgctgatgtactgacaagcctcgcgtacccgattatccatcggtggatggagcgactcgttaatcgcttccatgcgccgcagtaacaattgctcaagcagatttatcgccagcagctccgaatagcgcccttccccttgcccggcgttaatgatttgcccaaacaggtcgctgaaatgcggctggtgcgcttcatccgggcgaaagaaccccgtattggcaaatattgacggccagttaagccattcatgccagtaggcgcgcggacgaaagtaaacccactggtgataccattcgcgagcctccggatgacgaccgtagtgatgaatctctcctggcgggaacagcaaaatatcacccggtcggcaaacaaattctcgtccctgatttttcaccaccccctgaccgcgaatggtgagattgagaatataacctttcattcccagcggtcggtcgataaaaaaatcgagataaccgttggcctcaatcggcgttaaacccgccaccagatgggcattaaacgagtatcccggcagcaggggatcattttgcgcttcagccatacttttcatactcccgccattcag

SEQ ID NO: 31 - DNA, 27 bp, Artificial Sequence
  amorce fwd
gaggaaggatccatgggcattaaactg

SEQ ID NO: 32 - DNA, 24 bp, Artificial Sequence
  amorce rev
gctgcagatgaattcttaatggtg

SEQ ID NO: 33 - DNA, 28 bp, Artificial Sequence
  amorce Uhgb fw
caccatgagtatgagtagcaaagttatt

SEQ ID NO: 34 - DNA, 27 bp, Artificial Sequence
  amorce Uhgb rev
gatgatgcttgtacgtttggtaaattc

SEQ ID NO: 35 - DNA, 35 bp, Artificial Sequence
  amorce Fw
gaggaattaaccatgctgagcgtggaaaaacgctg

SEQ ID NO: 36 - DNA, 41 bp, Artificial Sequence
  amorce rev
agctgcagatctcgatcagtggtggtggtggtggtgctcga

SEQ ID NO: 37 - DNA, 5175 bp, Artificial Sequence
  pBAD- beta-1,3-mannooligosaccharide phosphorylase
aagaaaccaattgtccatattgcatcagacattgccgtcactgcgtcttttactggctcttctcgctaaccaaaccggtaaccccgcttattaaaagcattctgtaacaaagcgggaccaaagccatgacaaaaacgcgtaacaaaagtgtctataatcacggcagaaaagtccacattgattatttgcacggcgtcacactttgctatgccatagcatttttatccataagattagcggatcctacctgacgctttttatcgcaactctctactgtttctccatacccgttttttgggctaacaggaggaattaaccatgctgagcgtggaaaaacgctgtattctgagtccggtgccgggtagcccgtgggctggtaaaatggttctgaatccggcaatgattgcagatccggaagatccggaaaaaattcacatgctgtttcgtgccaccggcccgtggccgcaggctcgtttaccggaacgtccgctgccgtatccgatttttctgggttatggtgtgagttgcaatggcggtgcagattggcagtttgatctgagtcgtccggcaatggcaccgcgcctggaatttgatcgcgatcgctttctggcacgcggcatgcgtgatggcgtgatgtttgattatgcaaatggttgtattgaggatccgcgtctgttttattttgaagaacagctgtatctgagtgtggcatgtcgcgcatttccgccgggtccgtattgggaaaaagatgatccggttcagtgcatgccggaatgggcattcaaactgaatccggccgttcgcgaaaatagcaccgttaccatgctgtatcgcgttgatctggccgcactggcagccggccgctatgctgaagcctttagcccggttggtccgctgcatgatccggatctgagtgatgatcgtgatgcaatgctgtttccgcgtcgcctggaaattggcggtaaacgcaaaattgcctgcctgcatcgtccgaaacagccgtggaattatgcctgcggtaaagaagccgccgcaccgagcatttttctggcctttggcgatgaactgagcgattttcataccggtaaagcccgtacccagctgtttgccggtccggcctttgcccatgaagccaatcgcgtgggtgcaagttgggcaccgctggaactggaaccgggcctgtggctgctgccgtatcatggcaaacaggatgatcgtgttggttatacccagaattttatgctgctgcgcgaaaatggccgccaggccccggatattattgcacgcccggccgaacgcctgctgtatgccaccgaaccgtgggaactggaaggcgaattcactattccgtgtctgtttacctgtagtggtctgctgcgcccggatggcaccctgctgatgggttatggcgccgccgatcgtaaagttggcctggccagcattcgtctggaagaactgctggccgtgctgcgtccgctcgagcaccaccaccaccaccactgatcgagatctgcagctggtaccatatgggaattcgaagcttggctgttttggcggatgagagaagattttcagcctgatacagattaaatcagaacgcagaagcggtctgataaaacagaatttgcctggcggcagtagcgcggtggtcccacctgaccccatgccgaactcagaagtgaaacgccgtagcgccgatggtagtgtggggtctccccatgcgagagtagggaactgccaggcatcaaataaaacgaaaggctcagtcgaaagactgggcctttcgttttatctgttgtttgtcggtgaacgctctcctgagtaggacaaatccgccgggagcggatttgaacgttgcgaagcaacggcccggagggtggcgggcaggacgcccgccataaactgccaggcatcaaattaagcagaaggccatcctgacggatggcctttttgcgtttctacaaactcttttgtttatttttctaaatacattcaaatatgtatccgctcatgagacaataaccctgataaatgcttcaataatattgaaaaaggaagagtatgagtattcaacatttccgtgtcgcccttattcccttttttgcggcattttgccttcctgtttttgctcacccagaaacgctggtgaaagtaaaagatgctgaagatcagttgggtgcacgagtgggttacatcgaactggatctcaacagcggtaagatccttgagagttttcgccccgaagaacgttttccaatgatgagcacttttaaagttctgctatgtggcgcggtattatcccgtgttgacgccgggcaagagcaactcggtcgccgcatacactattctcagaatgacttggttgagtactcaccagtcacagaaaagcatcttacggatggcatgacagtaagagaattatgcagtgctgccataaccatgagtgataacactgcggccaacttacttctgacaacgatcggaggaccgaaggagctaaccgcttttttgcacaacatgggggatcatgtaactcgccttgatcgttgggaaccggagctgaatgaagccataccaaacgacgagcgtgacaccacgatgcctgtagcaatggcaacaacgttgcgcaaactattaactggcgaactacttactctagcttcccggcaacaattaatagactggatggaggcggataaagttgcaggaccacttctgcgctcggcccttccggctggctggtttattgctgataaatctggagccggtgagcgtgggtctcgcggtatcattgcagcactggggccagatggtaagccctcccgtatcgtagttatctacacgacggggagtcaggcaactatggatgaacgaaatagacagatcgctgagataggtgcctcactgattaagcattggtaactgtcagaccaagtttactcatatatactttagattgatttaaaacttcatttttaatttaaaaggatctaggtgaagatcctttttgataatctcatgaccaaaatcccttaacgtgagttttcgttccactgagcgtcagaccccgtagaaaagatcaaaggatcttcttgagatcctttttttctgcgcgtaatctgctgcttgcaaacaaaaaaaccaccgctaccagcggtggtttgtttgccggatcaagagctaccaactctttttccgaaggtaactggcttcagcagagcgcagataccaaatactgtccttctagtgtagccgtagttaggccaccacttcaagaactctgtagcaccgcctacatacctcgctctgctaatcctgttaccagtggctgctgccagtggcgataagtcgtgtcttaccgggttggactcaagacgatagttaccggataaggcgcagcggtcgggctgaacggggggttcgtgcacacagcccagcttggagcgaacgacctacaccgaactgagatacctacagcgtgagctatgagaaagcgccacgcttcccgaagggagaaaggcggacaggtatccggtaagcggcagggtcggaacaggagagcgcacgagggagcttccagggggaaacgcctggtatctttatagtcctgtcgggtttcgccacctctgacttgagcgtcgatttttgtgatgctcgtcaggggggcggagcctatggaaaaacgccagcaacgcggcctttttacggttcctggccttttgctggccttttgctcacatgttctttcctgcgttatcccctgattctgtggataaccgtattaccgcctttgagtgagctgataccgctcgccgcagccgaacgaccgagcgcagcgagtcagtgagcgaggaagcggaagagcgcctgatgcggtattttctccttacgcatctgtgcggtatttcacaccgcatatggtgcactctcagtacaatctgctctgatgccgcatagttaagccagtatacactccgctatcgctacgtgactgggtcatggctgcgccccgacacccgccaacacccgctgacgcgccctgacgggcttgtctgctcccggcatccgcttacagacaagctgtgaccgtctccgggagctgcatgtgtcagaggttttcaccgtcatcaccgaaacgcgcgaggcagcagatcaattcgcgcgcgaaggcgaagcggcatgcataatgtgcctgtcaaatggacgaagcagggattctgcaaaccctatgctactccgtcaagccgtcaattgtctgattcgttaccaattatgacaacttgacggctacatcattcactttttcttcacaaccggcacggaactcgctcgggctggccccggtgcattttttaaatacccgcgagaaatagagttgatcgtcaaaaccaacattgcgaccgacggtggcgataggcatccgggtggtgctcaaaagcagcttcgcctggctgatacgttggtcctcgcgccagcttaagacgctaatccctaactgctggcggaaaagatgtgacagacgcgacggcgacaagcaaacatgctgtgcgacgctggcgatatcaaaattgctgtctgccaggtgatcgctgatgtactgacaagcctcgcgtacccgattatccatcggtggatggagcgactcgttaatcgcttccatgcgccgcagtaacaattgctcaagcagatttatcgccagcagctccgaatagcgcccttccccttgcccggcgttaatgatttgcccaaacaggtcgctgaaatgcggctggtgcgcttcatccgggcgaaagaaccccgtattggcaaatattgacggccagttaagccattcatgccagtaggcgcgcggacgaaagtaaacccactggtgataccattcgcgagcctccggatgacgaccgtagtgatgaatctctcctggcgggaacagcaaaatatcacccggtcggcaaacaaattctcgtccctgatttttcaccaccccctgaccgcgaatggtgagattgagaatataacctttcattcccagcggtcggtcgataaaaaaatcgagataaccgttggcctcaatcggcgttaaacccgccaccagatgggcattaaacgagtatcccggcagcaggggatcattttgcgcttcagccatacttttcatactcccgccattcagag

SEQ ID NO: 38 - DNA, 6505 bp, Artificial Sequence
  pBAD-ACL0729 6505 bp
aagaaaccaattgtccatattgcatcagacattgccgtcactgcgtcttttactggctcttctcgctaaccaaaccggtaaccccgcttattaaaagcattctgtaacaaagcgggaccaaagccatgacaaaaacgcgtaacaaaagtgtctataatcacggcagaaaagtccacattgattatttgcacggcgtcacactttgctatgccatagcatttttatccataagattagcggatcctacctgacgctttttatcgcaactctctactgtttctccatacccgttttttgggctaacaggaggaattaaccatgggccaccaccaccaccatcacaaaaaaaaacaaagcatcaaaaagaactacggccaatacctgccactgtacaacctgggccaattaaaaagcagcatcacccccttcttcggcggcgatattaaaaccgaccaccaccactacctgttagaaccgaccaccgaaaacgatttatatgccaaccatatgagccgtaatattatttttaccatcgacgacgaaatgtactttctgaatggtaacacctatctgcagcagaatgatgagctgcaagttgaatatgacctgctgtatcagcgcgttgttagaagcaataccctgtttagcatcgaaagcctgtcctttattcccctgcatgacaacctggaattattagaagtgaccatcaaaaatacctccaataaaaatctgacccttgatgttattaccgcaattcctatttatgcccgttcagcagataatattcgtgaccaccgtcatgttaccagcctgctgaataaagttgaaatcaatgaacagaccgtgctggttaaaccgaccctgagctttgacgaacgtgggcatcatctgaatcatgaagcgtataccgtttctgcatatagcccgaccaccaaagtaaatcgcatcatcaccagcttagaagattttattgacggcggtagctttaattttcctaaaggtatttaccgtaaggattttgaaccaaagcctggatatgaggttatcggcgcaattggttttgaaccgtttattctgaaaccggaggagaccgcaacatttaatattagcatgggcatttttaaccagaatgaagatgcactgcacattattaacaaatataagacaaagaagagcgtggaagaagcgtttaaacacatgagaaattatttcgaagccgaaagcagcaaattaagcattagcatggttaataaggacgttgaactgctgctgcggtgggtgcgctttcagccggttctgcgtcgtatctttggtaacagctacctgccgcatcatgattatggccgtggcggtcgtggatggcgggacttatggcaggatttattaagcttaattctgattaacgacgagagtgttgaaacactgttatttaataacttccagggtattcgtatcgacggtagcaatgcaacaattattggtgataagccgggtgagtttctggcagatcgcaataaaatcgttagagtttggagcgaccacggtgcctggccgctgttaacaaccctgagctatattcatagcacgggacacattgaatttctgtttaaacagcagacctattttcatgaccaatttacccactataccaataaaaccagagatattgaaaccagcgaacatatattacgtgtgcacaacaaaccgtacttagggaccattctggaacatttactgctgcagaacattgttgcacactttaataccggcaaatttggctttgtgcggctggaaaatgcagattggaatgatggtctggacatggccaaaaataatggtgaaacaattgcatttacccatttctacgcaagcaatctgatgaaaatggcagaggtgatcgaaaaaatcaaccgtccggtgcgtctgtttaaaagcctgtacgatctgatctttgaaacaatcgacctgaagaccttttttgataatgttagcgatttcaaggacaccaccgttgaagtggacgcaaccaaattaagctatcaactggtagaactgtataaaaaacgcattgatcacattaacgagaatgcatggattaaagacacccacctgcagagctatatcaccgatagcaatgtttttctggacaccgcagataccatgaatctgaccggtcaagcaatggcactgttaaacgaaaccctgaccatgagccaggcaaaaagcgtcgcagataccaccaaaaaactgctgtttaataaagataacggcggttaccacctgaatagcaattaccataaaataatgatggacatgggccgtgcatttggatttagttacaaccataaagaaaacggcgcagtgttttctcatatggcaataatgtatgtttacggcctttataattacaaccttgttcagctgggtaatgagggttataaaagcttaattatgcgtgccattcatccggacgcacatacggttctgggtattccggaatactttaccgataaaggtgtcggtaagtatttatatcttactggtagcgcaagttggctgctgaaactgctgcaagagcaggtttttggtattacattttattacgggaagctgacgctgaatccgaagctggttcgtgaagattttatcaatcatcgcgcgagcattcagacgtttattcatggtaaattaatcaagatcacctacattaacctgaaaaatctggactatggcgcatacaaaatcgataaggttctgtatcagggtcaaccgattaatatagaacatacaaagatcgaaggggatattgaagtgtacctggatgaactgtaactcgagatctgcagctggtaccatatgggaattcgaagcttggctgttttggcggatgagagaagattttcagcctgatacagattaaatcagaacgcagaagcggtctgataaaacagaatttgcctggcggcagtagcgcggtggtcccacctgaccccatgccgaactcagaagtgaaacgccgtagcgccgatggtagtgtggggtctccccatgcgagagtagggaactgccaggcatcaaataaaacgaaaggctcagtcgaaagactgggcctttcgttttatctgttgtttgtcggtgaacgctctcctgagtaggacaaatccgccgggagcggatttgaacgttgcgaagcaacggcccggagggtggcgggcaggacgcccgccataaactgccaggcatcaaattaagcagaaggccatcctgacggatggcctttttgcgtttctacaaactcttttgtttatttttctaaatacattcaaatatgtatccgctcatgagacaataaccctgataaatgcttcaataatattgaaaaaggaagagtatgagtattcaacatttccgtgtcgcccttattcccttttttgcggcattttgccttcctgtttttgctcacccagaaacgctggtgaaagtaaaagatgctgaagatcagttgggtgcacgagtgggttacatcgaactggatctcaacagcggtaagatccttgagagttttcgccccgaagaacgttttccaatgatgagcacttttaaagttctgctatgtggcgcggtattatcccgtgttgacgccgggcaagagcaactcggtcgccgcatacactattctcagaatgacttggttgagtactcaccagtcacagaaaagcatcttacggatggcatgacagtaagagaattatgcagtgctgccataaccatgagtgataacactgcggccaacttacttctgacaacgatcggaggaccgaaggagctaaccgcttttttgcacaacatgggggatcatgtaactcgccttgatcgttgggaaccggagctgaatgaagccataccaaacgacgagcgtgacaccacgatgcctgtagcaatggcaacaacgttgcgcaaactattaactggcgaactacttactctagcttcccggcaacaattaatagactggatggaggcggataaagttgcaggaccacttctgcgctcggcccttccggctggctggtttattgctgataaatctggagccggtgagcgtgggtctcgcggtatcattgcagcactggggccagatggtaagccctcccgtatcgtagttatctacacgacggggagtcaggcaactatggatgaacgaaatagacagatcgctgagataggtgcctcactgattaagcattggtaactgtcagaccaagtttactcatatatactttagattgatttaaaacttcatttttaatttaaaaggatctaggtgaagatcctttttgataatctcatgaccaaaatcccttaacgtgagttttcgttccactgagcgtcagaccccgtagaaaagatcaaaggatcttcttgagatcctttttttctgcgcgtaatctgctgcttgcaaacaaaaaaaccaccgctaccagcggtggtttgtttgccggatcaagagctaccaactctttttccgaaggtaactggcttcagcagagcgcagataccaaatactgtccttctagtgtagccgtagttaggccaccacttcaagaactctgtagcaccgcctacatacctcgctctgctaatcctgttaccagtggctgctgccagtggcgataagtcgtgtcttaccgggttggactcaagacgatagttaccggataaggcgcagcggtcgggctgaacggggggttcgtgcacacagcccagcttggagcgaacgacctacaccgaactgagatacctacagcgtgagctatgagaaagcgccacgcttcccgaagggagaaaggcggacaggtatccggtaagcggcagggtcggaacaggagagcgcacgagggagcttccagggggaaacgcctggtatctttatagtcctgtcgggtttcgccacctctgacttgagcgtcgatttttgtgatgctcgtcaggggggcggagcctatggaaaaacgccagcaacgcggcctttttacggttcctggccttttgctggccttttgctcacatgttctttcctgcgttatcccctgattctgtggataaccgtattaccgcctttgagtgagctgataccgctcgccgcagccgaacgaccgagcgcagcgagtcagtgagcgaggaagcggaagagcgcctgatgcggtattttctccttacgcatctgtgcggtatttcacaccgcatatggtgcactctcagtacaatctgctctgatgccgcatagttaagccagtatacactccgctatcgctacgtgactgggtcatggctgcgccccgacacccgccaacacccgctgacgcgccctgacgggcttgtctgctcccggcatccgcttacagacaagctgtgaccgtctccgggagctgcatgtgtcagaggttttcaccgtcatcaccgaaacgcgcgaggcagcagatcaattcgcgcgcgaaggcgaagcggcatgcataatgtgcctgtcaaatggacgaagcagggattctgcaaaccctatgctactccgtcaagccgtcaattgtctgattcgttaccaattatgacaacttgacggctacatcattcactttttcttcacaaccggcacggaactcgctcgggctggccccggtgcattttttaaatacccgcgagaaatagagttgatcgtcaaaaccaacattgcgaccgacggtggcgataggcatccgggtggtgctcaaaagcagcttcgcctggctgatacgttggtcctcgcgccagcttaagacgctaatccctaactgctggcggaaaagatgtgacagacgcgacggcgacaagcaaacatgctgtgcgacgctggcgatatcaaaattgctgtctgccaggtgatcgctgatgtactgacaagcctcgcgtacccgattatccatcggtggatggagcgactcgttaatcgcttccatgcgccgcagtaacaattgctcaagcagatttatcgccagcagctccgaatagcgcccttccccttgcccggcgttaatgatttgcccaaacaggtcgctgaaatgcggctggtgcgcttcatccgggcgaaagaaccccgtattggcaaatattgacggccagttaagccattcatgccagtaggcgcgcggacgaaagtaaacccactggtgataccattcgcgagcctccggatgacgaccgtagtgatgaatctctcctggcgggaacagcaaaatatcacccggtcggcaaacaaattctcgtccctgatttttcaccaccccctgaccgcgaatggtgagattgagaatataacctttcattcccagcggtcggtcgataaaaaaatcgagataaccgttggcctcaatcggcgttaaacccgccaccagatgggcattaaacgagtatcccggcagcaggggatcattttgcgcttcagccatacttttcatactcccgccattcagag

SEQ ID NO: 39 - DNA, 70 bp, Artificial Sequence
  amorce FW
atgagcacagaaaaagaaaagatgattgctggtgagttgtatcgctcggcgtgtaggctggagctgcttc

SEQ ID NO: 40 - DNA, 70 bp, Artificial Sequence
  amorce RV
ttacaattttttaattattctggctggattaccgcccacgacaacgttgtcatatgaatatcctccttag

SEQ ID NO: 41 - DNA, 24 bp, Artificial Sequence
  amorce fw
gatgattgctggtgagttgtatcg

SEQ ID NO: 42 - DNA, 24 bp, Artificial Sequence
  amorce rv
ttaattattctggctggattaccg

SEQ ID NO: 43 - DNA, 70 bp, Artificial Sequence
  amorce FW
attatgcgcagcacagccactctccattcaggttcatccaaacaaacacagtgtaggctggagctgcttc

SEQ ID NO: 44 - DNA, 70 bp, Artificial Sequence
  amorce RV
acacgcgctaaacggccgtggcctttgacagtcaccggtgattcgttggccatatgaatatcctccttag

SEQ ID NO: 45 - DNA, 23 bp, Artificial Sequence
  amorce FW
gtgcgggtctgacgcctaaatac

SEQ ID NO: 46 - DNA, 23 bp, Artificial Sequence
  amorce rv
gatgggtttcaatcttcttgcct

SEQ ID NO: 47 - DNA, 40 bp, Artificial Sequence
  amorce FW
aaataggcgctcacgattaaaaggaagctgagttggctgc

SEQ ID NO: 48 - DNA, 40 bp, Artificial Sequence
  amorce RV
tagctttgcactgtttcagagtgaagacgaaagggcctcg

SEQ ID NO: 49 - DNA, 40 bp, Artificial Sequence
  amorce FW
cgaggccctttcgtcttcactctgaaacagtgcaaagcta

SEQ ID NO: 50 - DNA, 40 bp, Artificial Sequence
  amorce RV
tgttttttagcgtcaggcatctctaggattcctccggttc

SEQ ID NO: 51 - DNA, 40 bp, Artificial Sequence
  amorce FW
gaaccggaggaatcctagagatgcctgacgctaaaaaaca

SEQ ID NO: 52 - DNA, 40 bp, Artificial Sequence
  amorce RV
gcagccaactcagcttccttttaatcgtgagcgcctattt

SEQ ID NO: 53 - DNA, 20 bp, Artificial Sequence
  amorce FW
tctgaaacagtgcaaagcta

SEQ ID NO: 54 - DNA, 20 bp, Artificial Sequence
  amorce RV
ttaatcgtgagcgcctattt

SEQ ID NO: 55 - DNA, 5080 bp, Artificial Sequence
  sequence plasmidique du vecteur pBAD- Lin0857
aagaaaccaattgtccatattgcatcagacattgccgtcactgcgtcttttactggctcttctcgctaaccaaaccggtaaccccgcttattaaaagcattctgtaacaaagcgggaccaaagccatgacaaaaacgcgtaacaaaagtgtctataatcacggcagaaaagtccacattgattatttgcacggcgtcacactttgctatgccatagcatttttatccataagattagcggatcctacctgacgctttttatcgcaactctctactgtttctccatacccgttttttgggctaacaggaggaattaaccatggggaatatctatcgctacgaagaaaatccgcttattactccgttggatgtgaagcctattcatgagggatttgaagtgatcggcgcctttaacggcggtgtcgcggaatacaatggtgaagttctgctgctgctgcgcgtcgccgaaaaaccggttagcgaagatcccgaaatcgttctggcgccagtgtataatgctaagaataaagaattagaactgcaaagtttccgcctggacgatgaaaactacgacttcgaagatccgcgtatgattcgtagcaaagcgaaattggaaggatttagctatttgacctcgctcagttatatccgcatcgcgcgctcaaaagacggccaccacttcacactggatgaaaagccattcctgtatccattcaatgaatatcagaccttcggtattgaggacgctcgcgttacccaaattggagatacgtaccatgtgaacttttctgcggtctcagagtttggcgtcgctgatgccttggtgacgactaaggactttgaaaatctggaataccagggcaacatctttgcaccagaaaacaaagatgtactcatcttcccagaaaaaatcaatggtaagtattacgcgcttcaccggcccagcctcaaaagtattggcaatctggacatctggatcgcaagctcaccggacctgcggtccttcggcgatcatcgccatctcctcggtatccgtccgggcgaatatgattctggccgggtgggtggcggatgtgtgccgattaaaacagaagaaggctggttgattttgtaccacggagccaccgaagaaaatcgttatgtgatgggtgccgctttgctggatttgaatgatccaacaatcgtgttaaagcgcacgaaaactccgattctggagccggtagctgattacgagaaaaatggcttttttggcgatgtcgtttttgcctgtggtgcgatccaggaaggtgataccttacatatgtactacggcgtcgcggatacttcgatggctggctgcgatatgaagattagcgagattctccatcagttagaggttgaggcgaaacaccatcaccatcaccattaactcgagatctgcagctggtaccatatgggaattcgaagcttggctgttttggcggatgagagaagattttcagcctgatacagattaaatcagaacgcagaagcggtctgataaaacagaatttgcctggcggcagtagcgcggtggtcccacctgaccccatgccgaactcagaagtgaaacgccgtagcgccgatggtagtgtggggtctccccatgcgagagtagggaactgccaggcatcaaataaaacgaaaggctcagtcgaaagactgggcctttcgttttatctgttgtttgtcggtgaacgctctcctgagtaggacaaatccgccgggagcggatttgaacgttgcgaagcaacggcccggagggtggcgggcaggacgcccgccataaactgccaggcatcaaattaagcagaaggccatcctgacggatggcctttttgcgtttctacaaactcttttgtttatttttctaaatacattcaaatatgtatccgctcatgagacaataaccctgataaatgcttcaataatattgaaaaaggaagagtatgagtattcaacatttccgtgtcgcccttattcccttttttgcggcattttgccttcctgtttttgctcacccagaaacgctggtgaaagtaaaagatgctgaagatcagttgggtgcacgagtgggttacatcgaactggatctcaacagcggtaagatccttgagagttttcgccccgaagaacgttttccaatgatgagcacttttaaagttctgctatgtggcgcggtattatcccgtgttgacgccgggcaagagcaactcggtcgccgcatacactattctcagaatgacttggttgagtactcaccagtcacagaaaagcatcttacggatggcatgacagtaagagaattatgcagtgctgccataaccatgagtgataacactgcggccaacttacttctgacaacgatcggaggaccgaaggagctaaccgcttttttgcacaacatgggggatcatgtaactcgccttgatcgttgggaaccggagctgaatgaagccataccaaacgacgagcgtgacaccacgatgcctgtagcaatggcaacaacgttgcgcaaactattaactggcgaactacttactctagcttcccggcaacaattaatagactggatggaggcggataaagttgcaggaccacttctgcgctcggcccttccggctggctggtttattgctgataaatctggagccggtgagcgtgggtctcgcggtatcattgcagcactggggccagatggtaagccctcccgtatcgtagttatctacacgacggggagtcaggcaactatggatgaacgaaatagacagatcgctgagataggtgcctcactgattaagcattggtaactgtcagaccaagtttactcatatatactttagattgatttaaaacttcatttttaatttaaaaggatctaggtgaagatcctttttgataatctcatgaccaaaatcccttaacgtgagttttcgttccactgagcgtcagaccccgtagaaaagatcaaaggatcttcttgagatcctttttttctgcgcgtaatctgctgcttgcaaacaaaaaaaccaccgctaccagcggtggtttgtttgccggatcaagagctaccaactctttttccgaaggtaactggcttcagcagagcgcagataccaaatactgtccttctagtgtagccgtagttaggccaccacttcaagaactctgtagcaccgcctacatacctcgctctgctaatcctgttaccagtggctgctgccagtggcgataagtcgtgtcttaccgggttggactcaagacgatagttaccggataaggcgcagcggtcgggctgaacggggggttcgtgcacacagcccagcttggagcgaacgacctacaccgaactgagatacctacagcgtgagctatgagaaagcgccacgcttcccgaagggagaaaggcggacaggtatccggtaagcggcagggtcggaacaggagagcgcacgagggagcttccagggggaaacgcctggtatctttatagtcctgtcgggtttcgccacctctgacttgagcgtcgatttttgtgatgctcgtcaggggggcggagcctatggaaaaacgccagcaacgcggcctttttacggttcctggccttttgctggccttttgctcacatgttctttcctgcgttatcccctgattctgtggataaccgtattaccgcctttgagtgagctgataccgctcgccgcagccgaacgaccgagcgcagcgagtcagtgagcgaggaagcggaagagcgcctgatgcggtattttctccttacgcatctgtgcggtatttcacaccgcatatggtgcactctcagtacaatctgctctgatgccgcatagttaagccagtatacactccgctatcgctacgtgactgggtcatggctgcgccccgacacccgccaacacccgctgacgcgccctgacgggcttgtctgctcccggcatccgcttacagacaagctgtgaccgtctccgggagctgcatgtgtcagaggttttcaccgtcatcaccgaaacgcgcgaggcagcagatcaattcgcgcgcgaaggcgaagcggcatgcataatgtgcctgtcaaatggacgaagcagggattctgcaaaccctatgctactccgtcaagccgtcaattgtctgattcgttaccaattatgacaacttgacggctacatcattcactttttcttcacaaccggcacggaactcgctcgggctggccccggtgcattttttaaatacccgcgagaaatagagttgatcgtcaaaaccaacattgcgaccgacggtggcgataggcatccgggtggtgctcaaaagcagcttcgcctggctgatacgttggtcctcgcgccagcttaagacgctaatccctaactgctggcggaaaagatgtgacagacgcgacggcgacaagcaaacatgctgtgcgacgctggcgatatcaaaattgctgtctgccaggtgatcgctgatgtactgacaagcctcgcgtacccgattatccatcggtggatggagcgactcgttaatcgcttccatgcgccgcagtaacaattgctcaagcagatttatcgccagcagctccgaatagcgcccttccccttgcccggcgttaatgatttgcccaaacaggtcgctgaaatgcggctggtgcgcttcatccgggcgaaagaaccccgtattggcaaatattgacggccagttaagccattcatgccagtaggcgcgcggacgaaagtaaacccactggtgataccattcgcgagcctccggatgacgaccgtagtgatgaatctctcctggcgggaacagcaaaatatcacccggtcggcaaacaaattctcgtccctgatttttcaccaccccctgaccgcgaatggtgagattgagaatataacctttcattcccagcggtcggtcgataaaaaaatcgagataaccgttggcctcaatcggcgttaaacccgccaccagatgggcattaaacgagtatcccggcagcaggggatcattttgcgcttcagccatacttttcatactcccgccattcagag

SEQ ID NO: 56 - DNA, 72 bp, Artificial Sequence
  amorce fw
gcacaataacatcattcttcctgatcacgtttcaccgcagattatcatcaagattgcagcattacacgtctt

SEQ ID NO: 57 - DNA, 77 bp, Artificial Sequence
  amorce rev
tgtgggtttccgcgaactgctgccacgggttagctttgcactgtttcagatccatatgaatatcctccttagttcct

SEQ ID NO: 58 - DNA, 77 bp, Artificial Sequence
  amorce fw
aggaactaaggaggatattcatatggatctgaaacagtgcaaagctaacccgtggcagcagttcgcggaaacccaca

SEQ ID NO: 59 - DNA, 72 bp, Artificial Sequence
  amorce rev
aaaaacgtcattgccttgtttgaccgcccctgttttttagcgtcaggcatctctaggattcctccggttcct

SEQ ID NO: 60 - DNA, 29 bp, Artificial Sequence
  amorce fw
gcacaataacatcattcttcctgatcacg

SEQ ID NO: 61 - DNA, 26 bp, Artificial Sequence
  amorce rev
aaaaacgtcattgccttgtttgaccg

SEQ ID NO: 62 - DNA, 24 bp, Artificial Sequence
  amorce fw
cagcctgtctgttcgtgcgaaaga

SEQ ID NO: 63 - DNA, 19 bp, Artificial Sequence
  amorce rev
tcagagaggtacagcggtg

SEQ ID NO: 64 - DNA, 20 bp, Artificial Sequence
  amorce pBAB-fw
atgccatagcatttttatcc

SEQ ID NO: 65 - DNA, 18 bp, Artificial Sequence
  amorce pBAD-rev
gatttaatctgtatcagg

SEQ ID NO: 66 - DNA, 799 bp, Artificial Sequence
  promoteur IHF
tctgaaacagtgcaaagctaacccgtggcagcagttcgcggaaacccacaacaagggcgaccgtgttgaaggtaaaatcaagtctatcactgacttcggtatcttcatcggcttggacggcggcatcgacggcctggttcacctgtctgacatctcctggaacgttgcaggcgaagaagcagttcgtgaatacaaaaaaggcgacgaaatcgctgcagttgttctgcaggttgacgcagaacgtgaacgtatctccctgggcgttaaacagctcgcagaagatccgttcaacaactgggttgctctgaacaagaaaggcgctatcgtaaccggtaaagtaactgcagttgacgctaaaggcgcaaccgtagaactggctgacggcgttgaaggttacctgcgtgcttctgaagcatcccgtgaccgcgttgaagacgctaccctggttctgagcgttggcgacgaagttgaagctaaattcaccggcgttgatcgtaaaaaccgcgcaatcagcctgtctgttcgtgcgaaagacgaagctgacgagaaagatgcaatcgcaactgttaacaaacaggaagatgcaaacttctccaacaacgcaatggctgaagctttcaaagcagctaaaggcgagtaattctctgactcttcgggatttttattccgaagtttgttgagtttacttgacagattgcaggtttcgtcctgtaatcaagcactaagggcggctacggccgcccttaatcaatgcagcaacagcagccgcttaatttgcctttaaggaaccggaggaatc